European Patent Application EP 4 628 505 A1, published October 8, 2025. Title: 新型抗CTLA4抗体. Applicant: 嘉和生物药业有限公司. Application CN. The sequence listing filed with the application follows.

SEQUENCE LISTING (33 sequences)

SEQ ID NO: 1 - protein, 8 aa, synthetic construct
GRTASSNA

SEQ ID NO: 2 - protein, 8 aa, synthetic construct
ISATGGLT

SEQ ID NO: 3 - protein, 18 aa, synthetic construct
AVGRERWYLRHTENEYDY

SEQ ID NO: 4 - protein, 125 aa, synthetic construct
QVQLVESGGGLVEAGGSLRLSCATSGRTASSNAMAWFRQAPGKEREFVAAISATGGLTAYADSVKGRFTISRDNSKNAVYLQMNTLKPEDTAVYIGAVGRERWYLRHTENEYDYWGRGAQVTVSS

SEQ ID NO: 5 - protein, 357 aa, synthetic construct
QVQLVESGGGLVEAGGSLRLSCATSGRTASSNAMAWFRQAPGKEREFVAAISATGGLTAYADSVKGRFTISRDNSKNAVYLQMNTLKPEDTAVYIGAVGRERWYLRHTENEYDYWGRGAQVTVSSEPKSADKTHTCPPCPAPELLGGPSVFLFPPKPKDTLMISRTPEVTCVVVDVSHEDPEVKFNWYVDGVEVHNAKTKPREEQYNSTYRVVSVLTVLHQDWLNGKEYKCKVSNKALPAPIEKTISKAKGQPREPQVYTLPPSREEMTKNQVSLTCLVKGFYPSDIAVEWESNGQPENNYKTTPPVLDSDGSFFLYSKLTVDKSRWQQGNVFSCSVMHEALHNHYTQKSLSLSPGK

SEQ ID NO: 6 - DNA, 1074 bp, synthetic construct
  source 1..1074: mol_type = other DNA
caggtccagctcgtcgagtcaggcggcggcctcgtggaagccggaggaagtttgaggctctcctgcgcaacaagcggcaggaccgccagcagcaacgccatggcatggtttaggcaggcacccggcaaggagagggagttcgtggctgctatcagtgccacaggaggcttgacagcctacgccgactccgtgaagggaaggttcacaatcagcagagacaactccaagaacgcagtttacctgcagatgaacacactgaagcccgaggacaccgccgtgtatattggcgccgttggccgtgaaaggtggtacttgaggcacaccgagaacgaatacgactactggggcaggggcgcccaggtgaccgtctcttccgagcccaaatctgctgacaaaactcacacatgcccaccgtgcccagcacctgaactcctggggggaccgtcagtcttcctcttccccccaaaacccaaggacaccctcatgatctcccggacccccgaggtcacatgcgtggtggtggacgtgagccacgaagaccctgaggtcaagttcaactggtacgtggacggcgtggaggtgcataatgccaagacaaagccgcgggaggagcagtacaacagcacgtaccgtgtggtcagcgtcctcaccgtcctgcaccaggactggctgaatggcaaggagtacaagtgcaaggtctccaacaaagccctcccagcccccatcgagaaaaccatctccaaagccaaagggcagccccgagaaccacaggtgtacaccctgcccccatcccgggaggagatgaccaagaaccaggtcagcctgacctgcctggtcaaaggcttctatcccagcgacatcgccgtggagtgggagagcaatgggcagccggagaacaactacaagaccacgcctcccgtgctggactccgacggctccttcttcctctacagcaagctcaccgtggacaagagcaggtggcagcaggggaacgtcttctcatgctccgtgatgcatgaggctctgcacaaccactacacgcagaagagcctctccctgtctccgggtaaatga

SEQ ID NO: 7 - protein, 125 aa, synthetic construct
EVQLVESGGGLVQPGGSLRLSCAASGRTASSNAMAWVRQAPGKEREFVSAISATGGLTAYADSVKGRFTISRDNSKNTLYLQMNSLRAEDTAVYYCAVGRERWYLRHTENEYDYWGQGTLVTVSS

SEQ ID NO: 8 - protein, 357 aa, synthetic construct
EVQLVESGGGLVQPGGSLRLSCAASGRTASSNAMAWVRQAPGKEREFVSAISATGGLTAYADSVKGRFTISRDNSKNTLYLQMNSLRAEDTAVYYCAVGRERWYLRHTENEYDYWGQGTLVTVSSEPKSADKTHTCPPCPAPELLGGPSVFLFPPKPKDTLMISRTPEVTCVVVDVSHEDPEVKFNWYVDGVEVHNAKTKPREEQYNSTYRVVSVLTVLHQDWLNGKEYKCKVSNKALPAPIEKTISKAKGQPREPQVYTLPPSREEMTKNQVSLTCLVKGFYPSDIAVEWESNGQPENNYKTTPPVLDSDGSFFLYSKLTVDKSRWQQGNVFSCSVMHEALHNHYTQKSLSLSPGK

SEQ ID NO: 9 - DNA, 1074 bp, synthetic construct
  source 1..1074: mol_type = other DNA
gaggtgcagttggtggagagcgggggggggctggtgcagcctggaggaagtttgaggttgagctgtgccgcaagcgggaggacagccagtagcaacgcaatggcctgggtgaggcaggcacccggaaaggagagggagttcgtgagtgccatttccgccaccggtggactgaccgcctacgccgacagtgtgaaggggaggttcaccatctccagggacaacagcaagaacaccctgtacctgcagatgaacagcctgagggccgaggacacagccgtgtactactgcgcagttggcagggagcgctggtacttgaggcacaccgagaacgagtacgactactggggccagggcaccctggttaccgtgtcctccgagcccaaatctgctgacaaaactcacacatgcccaccgtgcccagcacctgaactcctggggggaccgtcagtcttcctcttccccccaaaacccaaggacaccctcatgatctcccggacccccgaggtcacatgcgtggtggtggacgtgagccacgaagaccctgaggtcaagttcaactggtacgtggacggcgtggaggtgcataatgccaagacaaagccgcgggaggagcagtacaacagcacgtaccgtgtggtcagcgtcctcaccgtcctgcaccaggactggctgaatggcaaggagtacaagtgcaaggtctccaacaaagccctcccagcccccatcgagaaaaccatctccaaagccaaagggcagccccgagaaccacaggtgtacaccctgcccccatcccgggaggagatgaccaagaaccaggtcagcctgacctgcctggtcaaaggcttctatcccagcgacatcgccgtggagtgggagagcaatgggcagccggagaacaactacaagaccacgcctcccgtgctggactccgacggctccttcttcctctacagcaagctcaccgtggacaagagcaggtggcagcaggggaacgtcttctcatgctccgtgatgcatgaggctctgcacaaccactacacgcagaagagcctctccctgtctccgggtaaatga

SEQ ID NO: 10 - protein, 125 aa, synthetic construct
EVQLVESGGGLVQPGGSLRLSCAASGRTASSNAMAWFRQAPGKEREFVSAISATGGLTAYADSVKGRFTISRDNSKNTLYLQMNSLRAEDTAVYIGAVGRERWYLRHTENEYDYWGQGTLVTVSS

SEQ ID NO: 11 - protein, 357 aa, synthetic construct
EVQLVESGGGLVQPGGSLRLSCAASGRTASSNAMAWFRQAPGKEREFVSAISATGGLTAYADSVKGRFTISRDNSKNTLYLQMNSLRAEDTAVYIGAVGRERWYLRHTENEYDYWGQGTLVTVSSEPKSADKTHTCPPCPAPELLGGPSVFLFPPKPKDTLMISRTPEVTCVVVDVSHEDPEVKFNWYVDGVEVHNAKTKPREEQYNSTYRVVSVLTVLHQDWLNGKEYKCKVSNKALPAPIEKTISKAKGQPREPQVYTLPPSREEMTKNQVSLTCLVKGFYPSDIAVEWESNGQPENNYKTTPPVLDSDGSFFLYSKLTVDKSRWQQGNVFSCSVMHEALHNHYTQKSLSLSPGK

SEQ ID NO: 12 - DNA, 1074 bp, synthetic construct
  source 1..1074: mol_type = other DNA
gaggtgcagttggtggagagcgggggggggctggtgcagcctggaggaagtttgaggttgagctgtgccgcaagcgggaggacagccagtagcaacgcaatggcctggtttaggcaggcacccggcaaggagagggagttcgtgagtgccatttccgccaccggtggactgacagcctacgccgacagtgtgaagggcaggttcaccatctccagggacaactccaagaacaccctgtacctgcagatgaacagcctgagggccgaggacaccgccgtgtacatcggagccgttggcagggagcgatggtacttgaggcacaccgagaacgagtacgactactggggccagggcaccctggtgaccgtgtccagcgagcccaaatctgctgacaaaactcacacatgcccaccgtgcccagcacctgaactcctggggggaccgtcagtcttcctcttccccccaaaacccaaggacaccctcatgatctcccggacccccgaggtcacatgcgtggtggtggacgtgagccacgaagaccctgaggtcaagttcaactggtacgtggacggcgtggaggtgcataatgccaagacaaagccgcgggaggagcagtacaacagcacgtaccgtgtggtcagcgtcctcaccgtcctgcaccaggactggctgaatggcaaggagtacaagtgcaaggtctccaacaaagccctcccagcccccatcgagaaaaccatctccaaagccaaagggcagccccgagaaccacaggtgtacaccctgcccccatcccgggaggagatgaccaagaaccaggtcagcctgacctgcctggtcaaaggcttctatcccagcgacatcgccgtggagtgggagagcaatgggcagccggagaacaactacaagaccacgcctcccgtgctggactccgacggctccttcttcctctacagcaagctcaccgtggacaagagcaggtggcagcaggggaacgtcttctcatgctccgtgatgcatgaggctctgcacaaccactacacgcagaagagcctctccctgtctccgggtaaatga

SEQ ID NO: 13 - protein, 10 aa, synthetic construct
GFTFSSYTMA

SEQ ID NO: 14 - protein, 17 aa, synthetic construct
GISRSGGTTNYGDSVKG

SEQ ID NO: 15 - protein, 4 aa, synthetic construct
VSDY

SEQ ID NO: 16 - protein, 113 aa, synthetic construct
QVQLVESGGGLVQPGGSLTLSCAASGFTFSSYTMAWYRQAPGKEREVVAGISRSGGTTNYGDSVKGRFTISRDNAKNTVYLQMNSLKPEDTAVYYCRAVSDYWGQGTQVTVSS

SEQ ID NO: 17 - protein, 345 aa, synthetic construct
QVQLVESGGGLVQPGGSLTLSCAASGFTFSSYTMAWYRQAPGKEREVVAGISRSGGTTNYGDSVKGRFTISRDNAKNTVYLQMNSLKPEDTAVYYCRAVSDYWGQGTQVTVSSEPKSADKTHTCPPCPAPELLGGPSVFLFPPKPKDTLMISRTPEVTCVVVDVSHEDPEVKFNWYVDGVEVHNAKTKPREEQYNSTYRVVSVLTVLHQDWLNGKEYKCKVSNKALPAPIEKTISKAKGQPREPQVYTLPPSREEMTKNQVSLTCLVKGFYPSDIAVEWESNGQPENNYKTTPPVLDSDGSFFLYSKLTVDKSRWQQGNVFSCSVMHEALHNHYTQKSLSLSPGK

SEQ ID NO: 18 - DNA, 1038 bp, synthetic construct
  source 1..1038: mol_type = other DNA
caggtgcagctggtggaaagtggcggcggcctggtgcagcccggaggaagcctgacactgtcctgcgccgcctccggttttaccttctcctcctacacaatggcctggtacaggcaggcacccggcaaggagagggaggtggtggctggcatttccagaagcggaggaaccacaaactacggggatagtgtgaagggcaggtttaccatttccagggacaacgccaagaacaccgtgtacctgcagatgaacagcctgaagcccgaggacaccgcagtgtactactgcagggccgtgagcgactactggggccaggggacccaggtgaccgtgagctccgagcccaaatctgctgacaaaactcacacatgcccaccgtgcccagcacctgaactcctggggggaccgtcagtcttcctcttccccccaaaacccaaggacaccctcatgatctcccggacccccgaggtcacatgcgtggtggtggacgtgagccacgaagaccctgaggtcaagttcaactggtacgtggacggcgtggaggtgcataatgccaagacaaagccgcgggaggagcagtacaacagcacgtaccgtgtggtcagcgtcctcaccgtcctgcaccaggactggctgaatggcaaggagtacaagtgcaaggtctccaacaaagccctcccagcccccatcgagaaaaccatctccaaagccaaagggcagccccgagaaccacaggtgtacaccctgcccccatcccgggaggagatgaccaagaaccaggtcagcctgacctgcctggtcaaaggcttctatcccagcgacatcgccgtggagtgggagagcaatgggcagccggagaacaactacaagaccacgcctcccgtgctggactccgacggctccttcttcctctacagcaagctcaccgtggacaagagcaggtggcagcaggggaacgtcttctcatgctccgtgatgcatgaggctctgcacaaccactacacgcagaagagcctctccctgtctccgggtaaatga

SEQ ID NO: 19 - protein, 113 aa, synthetic construct
EVQLLESGGGLVQPGGSLRLSCAASGFTFSSYTMAWYRQAPGKEREVVAGISRSGGTTNYGDSVKGRFTISRDNSKNTLYLQMNSLRAEDTAVYYCRAVSDYWGQGTLVTVSS

SEQ ID NO: 20 - protein, 345 aa, synthetic construct
EVQLLESGGGLVQPGGSLRLSCAASGFTFSSYTMAWYRQAPGKEREVVAGISRSGGTTNYGDSVKGRFTISRDNSKNTLYLQMNSLRAEDTAVYYCRAVSDYWGQGTLVTVSSEPKSADKTHTCPPCPAPELLGGPSVFLFPPKPKDTLMISRTPEVTCVVVDVSHEDPEVKFNWYVDGVEVHNAKTKPREEQYNSTYRVVSVLTVLHQDWLNGKEYKCKVSNKALPAPIEKTISKAKGQPREPQVYTLPPSREEMTKNQVSLTCLVKGFYPSDIAVEWESNGQPENNYKTTPPVLDSDGSFFLYSKLTVDKSRWQQGNVFSCSVMHEALHNHYTQKSLSLSPGK

SEQ ID NO: 21 - DNA, 1026 bp, synthetic construct
  source 1..1026: mol_type = other DNA
gaagtgcaactactagaaagtggtggtggtctcgtgcagcctggcggatctctgagactgtcttgtgctgcttctggcttcaccttctcctcctacaccatggcctggtatcgccaagcccccggaaaagagcgggaagtggtggccggcatctccagatccggcggcaccaccaactacggcgactccgtgaagggcagatttaccatctctcgggacaactccaagaacaccctgtacctgcagatgaatagcctgcgggccgaggatacagctgtgtactactgcagagccgtgtccgactactggggccagggcacactggtcaccgtgtctagcgataagacacacacctgccccccttgtcctgctcccgagctgctgggcggccctagcgtgttcctgtttccacccaagcctaaggacaccctgatgatctcccggacacccgaggtgacctgcgtggtggtggacgtgtctcacgaggatcctgaggtgaagttcaactggtatgtggatggcgtggaggtgcacaatgccaagaccaagcccagagaggagcagtacaactctacatatagggtggtgagcgtgctgaccgtgctgcaccaggactggctgaacggcaaggagtataagtgcaaggtgtccaataaggccctgcccgcccccatcgagaagacaatcagcaaggccaagggccagcctcgggagccacaggtgtacaccctgcctccatccagagacgagctgacaaagaaccaggtgtctctgacatgtctggtgaagggcttctatcctagcgatatcgccgtggagtgggagtccaatggccagccagagaacaattacaagaccacaccccctgtgctggactccgatggctccttctttctgtattccaagctgaccgtggataagtctcggtggcagcagggcaacgtgttcagctgttccgtgatgcacgaagccctgcataatcactatactcagaaatccctgtccctgtcacctggaaagtgataa

SEQ ID NO: 22 - protein, 10 aa, synthetic construct
GRTFSSYDMG

SEQ ID NO: 23 - protein, 17 aa, synthetic construct
AISWGGVNTYYADSVKG

SEQ ID NO: 24 - protein, 18 aa, synthetic construct
GSAPYSSSRSSAQETYAQ

SEQ ID NO: 25 - protein, 127 aa, synthetic construct
EVQLVESGGGLVQAGGSLRLSCLASGRTFSSYDMGWFRQAPGKEREFVAAISWGGVNTYYADSVKGRFTISRDNAKNTVYLQMNSLKPEDTAVYYCARGSAPYSSSRSSAQETYAQWGQGTQVTVSS

SEQ ID NO: 26 - protein, 359 aa, synthetic construct
EVQLVESGGGLVQAGGSLRLSCLASGRTFSSYDMGWFRQAPGKEREFVAAISWGGVNTYYADSVKGRFTISRDNAKNTVYLQMNSLKPEDTAVYYCARGSAPYSSSRSSAQETYAQWGQGTQVTVSSEPKSADKTHTCPPCPAPELLGGPSVFLFPPKPKDTLMISRTPEVTCVVVDVSHEDPEVKFNWYVDGVEVHNAKTKPREEQYNSTYRVVSVLTVLHQDWLNGKEYKCKVSNKALPAPIEKTISKAKGQPREPQVYTLPPSREEMTKNQVSLTCLVKGFYPSDIAVEWESNGQPENNYKTTPPVLDSDGSFFLYSKLTVDKSRWQQGNVFSCSVMHEALHNHYTQKSLSLSPGK

SEQ ID NO: 27 - DNA, 1087 bp, synthetic construct
  source 1..1087: mol_type = other DNA
gaggtgcagttggtggagagcgggggggggctggtgcaggctggaggaagtttgaggttgagctgtttggcttctgggaggacctttagcagctatgacatgggatggtttaggcaggcccccggaaaggagagggagttcgtggccgccatttcctgggggggggtgaatacctactacgctgactccgtgaagggacgattcacaatctcccgggacaacgccaagaacacagtgtatctgcagatgaacagcctcaagcctgaagacaccgctgtgtattattgcgcccggggctccgccccctattcctcttctaggtcctccgcccaggaaacctacgcccagtggggccagggcacccaggtcacagtgtcctccgagcccaaatctgctgacaaaactcacacatgcccaccgtgcccagcacctgaactcctggggggaccgtcagtcttcctcttccccccaaaacccaaggacaccctcatgatctcccggacccccgaggtcacatgcgtggtggtggacgtgagccacgaagaccctgaggtcaagttcaactggtacgtggacggcgtggaggtgcataatgccaagacaaagccgcgggaggagcagtacaacagcacgtaccgtgtggtcagcgtcctcaccgtcctgcaccaggactggctgaatggcaaggagtacaagtgcaaggtctccaacaaagccctcccagcccccatcgagaaaaccatctccaaagccaaagggcagccccgagaaccacaggtgtacaccctgcccccatcccgggaggagatgaccaagaaccaggtcagcctgacctgcctggtcaaaggcttctatcccagcgacatcgccgtggagtgggagagcaatgggcagccggagaacaactacaagaccacgcctcccgtgctggactccgacggctccttcttcctctacagcaagctcaccgtggacaagagcaggtggcagcaggggaacgtcttctcatgctccgtgatgcatgaggctctgcacaaccactacacgcagaagagcctctccctgtctccgggtaaatgattctaga

SEQ ID NO: 28 - protein, 127 aa, synthetic construct
EVQLVESGGGLVQPGGSLRLSCAASGRTFSSYDMGWFRQAPGKEREFVAAISWGGVNTYYADSVKGRFTISRDNAKNTLYLQMNSLRAEDTAVYYCARGSAPYSSSRSSAQETYAQWGQGTLVTVSS

SEQ ID NO: 29 - protein, 359 aa, synthetic construct
EVQLVESGGGLVQPGGSLRLSCAASGRTFSSYDMGWFRQAPGKEREFVAAISWGGVNTYYADSVKGRFTISRDNAKNTLYLQMNSLRAEDTAVYYCARGSAPYSSSRSSAQETYAQWGQGTLVTVSSEPKSADKTHTCPPCPAPELLGGPSVFLFPPKPKDTLMISRTPEVTCVVVDVSHEDPEVKFNWYVDGVEVHNAKTKPREEQYNSTYRVVSVLTVLHQDWLNGKEYKCKVSNKALPAPIEKTISKAKGQPREPQVYTLPPSREEMTKNQVSLTCLVKGFYPSDIAVEWESNGQPENNYKTTPPVLDSDGSFFLYSKLTVDKSRWQQGNVFSCSVMHEALHNHYTQKSLSLSPGK

SEQ ID NO: 30 - DNA, 1080 bp, synthetic construct
  source 1..1080: mol_type = other DNA
gaggtgcagctggtggagtccggaggaggactggtgcagcctggaggaagcctgaggctgtcctgcgctgcttccggaaggacctttagttcctatgatatggggtggttcaggcaggcccctggaaaagaaagggagttcgtggctgctatttcctgggggggcgtgaacacctactacgccgactccgtgaagggcaggttcaccatctccagggacaacgccaagaacaccctgtacctgcagatgaactccctgagggccgaggacaccgccgtgtactactgcgccaggggctccgccccctactcctcctccaggtcctccgcccaggagacatacgcccagtggggccagggcaccctggtgaccgtgtcctccgagcccaaatctgctgacaaaactcacacatgcccaccgtgcccagcacctgaactcctggggggaccgtcagtcttcctcttccccccaaaacccaaggacaccctcatgatctcccggacccccgaggtcacatgcgtggtggtggacgtgagccacgaagaccctgaggtcaagttcaactggtacgtggacggcgtggaggtgcataatgccaagacaaagccgcgggaggagcagtacaacagcacgtaccgtgtggtcagcgtcctcaccgtcctgcaccaggactggctgaatggcaaggagtacaagtgcaaggtctccaacaaagccctcccagcccccatcgagaaaaccatctccaaagccaaagggcagccccgagaaccacaggtgtacaccctgcccccatcccgggaggagatgaccaagaaccaggtcagcctgacctgcctggtcaaaggcttctatcccagcgacatcgccgtggagtgggagagcaatgggcagccggagaacaactacaagaccacgcctcccgtgctggactccgacggctccttcttcctctacagcaagctcaccgtggacaagagcaggtggcagcaggggaacgtcttctcatgctccgtgatgcatgaggctctgcacaaccactacacgcagaagagcctctccctgtctccgggtaaatga

SEQ ID NO: 31 - protein, 125 aa, synthetic construct
EVQLVESGGGLVQPGGSLRLSCAASGRTASSNAMAWFRQAPGKEREFVSAISATGGLTAYADSVKGRFTISRDNSKNTLYLQMNSLRAEDTAVYYCAVGRERWYLRHTENEYDYWGQGTLVTVSS

SEQ ID NO: 32 - protein, 357 aa, synthetic construct
EVQLVESGGGLVQPGGSLRLSCAASGRTASSNAMAWFRQAPGKEREFVSAISATGGLTAYADSVKGRFTISRDNSKNTLYLQMNSLRAEDTAVYYCAVGRERWYLRHTENEYDYWGQGTLVTVSSEPKSADKTHTCPPCPAPELLGGPSVFLFPPKPKDTLMISRTPEVTCVVVDVSHEDPEVKFNWYVDGVEVHNAKTKPREEQYNSTYRVVSVLTVLHQDWLNGKEYKCKVSNKALPAPIEKTISKAKGQPREPQVYTLPPSRDELTKNQVSLTCLVKGFYPSDIAVEWESNGQPENNYKTTPPVLDSDGSFFLYSKLTVDKSRWQQGNVFSCSVMHEALHNHYTQKSLSLSPGK

SEQ ID NO: 33 - DNA, 1074 bp, synthetic construct
  source 1..1074: mol_type = other DNA
gaagtgcagctggtggagagcggaggaggattggtgcagcctggaggaagcctgaggctgagttgtgccgctagtgggaggacagcaagtagtaacgcaatggcatggtttaggcaggcccccggaaaagagagggagttcgtgagcgccatttccgccaccggaggattgacagcctacgctgattccgtgaagggcaggttcaccatcagcagggacaactccaagaacacactgtacctgcagatgaacagcctgagggccgaggacacagccgtttactactgcgccgtgggcagggaaaggtggtacttgaggcacaccgagaacgagtacgactactggggccagggcaccttggtgacagtctcttccgagcctaaaagcgccgacaaaactcacacatgcccaccgtgcccagcacctgaactcctggggggaccgtcagtcttcctcttccccccaaaacccaaggacaccctcatgatctcccggacccccgaggtcacatgcgtggtggtggacgtgagccacgaagaccctgaggtcaagttcaactggtacgtggacggcgtggaggtgcataatgccaagacaaagccgcgggaggagcagtacaacagcacgtaccgtgtggtcagcgtcctcaccgtcctgcaccaggactggctgaatggcaaggagtacaagtgcaaggtctccaacaaagccctcccagcccccatcgagaaaaccatctccaaagccaaagggcagccccgagaaccacaggtgtacaccctgcccccatcccgggacgagctgaccaagaaccaggtcagcctgacctgcctggtcaaaggcttctatcccagcgacatcgccgtggagtgggagagcaatgggcagccggagaacaactacaagaccacgcctcccgtgctggactccgacggctccttcttcctctacagcaagctcaccgtggacaagagcaggtggcagcaggggaacgtcttctcatgctccgtgatgcatgaggctctgcacaaccactacacgcagaagagcctctccctgtctccgggtaaatga